European Patent Application EP 4 151 737 A1, published March 22, 2023. Title: Methods of selectively modulating the activity of distinct subtypes of cells. Applicant: Ecole Normale Superieure de Lyon. Application EP. The sequence listing filed with the application follows.

SEQUENCE LISTING (16 sequences)

SEQ ID NO: 1 - DNA, 2217 bp, synthetic construct
  misc_feature 1..2217: note = Truncated and mutated (Y481A, R533A, S548L, F549S) MV H protein(HcDelta18) fused to Designed Ankyrin Repeat Protein(DARPin)-29.2 specific for human CD4
  source 1..2217: mol_type = other DNA
  CDS 1..2217
atgggaagtaggatagtcattaacagagaacatcttatgattgatagaccttatgttttgctggctgttctgtttgtcatgtttctgagcttgatcgggttgctagccattgcaggaattcgacttcatcgggcagccatctacaccgcagagatccataaaagcctcagcaccaatctagatgtaactaactcaatcgagcatcaggtcaaggacgtgctgacaccactcttcaaaatcatcggtgatgaagtgggcctgaggacacctcagagattcactgacctagtgaaattcatctctgacaagattaaattccttaatccggatagggagtacgacttcagagatctcacttggtgtatcaacccgccagagagaatcaaattggattatgatcaatactgtgcagatgtggctgctgaagagctcatgaatgcattggtgaactcaactctactggagaccagaacaaccaatcagttcctagctgtctcaaagggaaactgctcagggcccactacaatcagaggtcaattctcaaacatgtcgctgtccctgttagacttgtatttaggtcgaggttacaatgtgtcatctatagtcactatgacatcccagggaatgtatgggggaacttacctagtggaaaagcctaatctgagcagcaaaaggtcagagttgtcacaactgagcatgtaccgagtgtttgaagtaggtgttatcagaaatccgggtttgggggctccggtgttccatatgacaaactatcttgagcaaccagtcagtaatgatctcagcaactgtatggtggctttgggggagctcaaactcgcagccctttgtcacggggaagattctatcacaattccctatcagggatcagggaaaggtgtcagcttccagctcgtcaagctaggtgtctggaaatccccaaccgacatgcaatcctgggtccccttatcaacggatgatccagtgatagacaggctttacctctcatctcacagaggtgttatcgctgacaaccaagcaaaatgggctgtcccgacaacacgaacagatgacaagttgcgaatggagacatgcttccaacaggcgtgtaagggtaaaatccaagcactctgcgagaatcccgagtgggcaccattgaaggataacaggattccttcatacggggtcttgtctgttgatctgagtctgacagttgagcttaaaatcaaaattgcttcgggattcgggccattgatcacacacggttcagggatggacctatacaaatccaaccacaacaatgtgtattggctgactatcccgccaatgaagaacctagccttaggtgtaatcaacacattggagtggataccgagattcaaggttagtcccgcactcttcactgtcccaattaaggaagcaggcggagactgccatgccccaacatacctacctgcggaggtggatggtgatgtcaaactcagttccaatctggtgattctacctggtcaagatctccaatatgttttggcaacctacgatacttccgcggttgaacatgctgtggtttattacgtttacagcccaagccgcctatcgtcttacttttatccttttaggttgcctataaagggggtccccatcgaattacaagtggaatgcttcacatgggaccaaaaactctggtgccgtcacttctgtgtgcttgcggactcagaatctggtggacatatcactcactctgggatggtgggcatgggagtcagctgcacagtcacccgggaagatggaaccaatgcggcccagccggccgacctgggtaagaaactgctggaagctgctcgtgctggtcaggacgacgaagttcgtatcctgatggctaacggtgctgacgttaacgctactgacactcttggtcgtactccgctacacctggctgctcagaatggtcacctggaaatcgttgaagttctgctgaagcacagtgctgacgttaacgctattgaagaggttggtatgactccgctgcacctggctgttgttgctggtcacctggaaatcgttgaagttctgctgaagaacggtgctgacgttaacgctcaggacaaattcggtaagaccgctttcgacatctccatcgactacggtaacgaggacctggctgaaatcctgcaaaagcttaatgcggccgcaagaggttctcatcaccatcaccatcactaa

SEQ ID NO: 2 - protein, 738 aa, synthetic construct
  REGION 1..738: note = Synthetic Construct
MGSRIVINREHLMIDRPYVLLAVLFVMFLSLIGLLAIAGIRLHRAAIYTAEIHKSLSTNLDVTNSIEHQVKDVLTPLFKIIGDEVGLRTPQRFTDLVKFISDKIKFLNPDREYDFRDLTWCINPPERIKLDYDQYCADVAAEELMNALVNSTLLETRTTNQFLAVSKGNCSGPTTIRGQFSNMSLSLLDLYLGRGYNVSSIVTMTSQGMYGGTYLVEKPNLSSKRSELSQLSMYRVFEVGVIRNPGLGAPVFHMTNYLEQPVSNDLSNCMVALGELKLAALCHGEDSITIPYQGSGKGVSFQLVKLGVWKSPTDMQSWVPLSTDDPVIDRLYLSSHRGVIADNQAKWAVPTTRTDDKLRMETCFQQACKGKIQALCENPEWAPLKDNRIPSYGVLSVDLSLTVELKIKIASGFGPLITHGSGMDLYKSNHNNVYWLTIPPMKNLALGVINTLEWIPRFKVSPALFTVPIKEAGGDCHAPTYLPAEVDGDVKLSSNLVILPGQDLQYVLATYDTSAVEHAVVYYVYSPSRLSSYFYPFRLPIKGVPIELQVECFTWDQKLWCRHFCVLADSESGGHITHSGMVGMGVSCTVTREDGTNAAQPADLGKKLLEAARAGQDDEVRILMANGADVNATDTLGRTPLHLAAQNGHLEIVEVLLKHSADVNAIEEVGMTPLHLAVVAGHLEIVEVLLKNGADVNAQDKFGKTAFDISIDYGNEDLAEILQKLNAAARGSHHHHHH

SEQ ID NO: 3 - DNA, 2529 bp, synthetic construct
  misc_feature 1..2529: note = Truncated and mutated (E501A, W504A, Q530A, E533A) NiV G protein(GcDelta34) fused to a single chain antibody directed to humanCD8 (scFvC8-Vh1) linked with an additional (G4S)3 linker
  source 1..2529: mol_type = other DNA
  CDS 1..2529
atgaagaagatcaacgagggcctgctggacagcaagatcctgagcgccttcaacaccgtgatcgccctgctgggcagcatcgtgatcattgtgatgaacatcatgatcatccagaactacaccagaagcaccgacaaccaggccgtgatcaaggacgctctccaggggatccagcagcagatcaagggcctggccgacaagatcggcaccgagatcggccccaaggtgtccctgatcgacaccagcagcaccatcaccatccccgccaacatcggcctgctggggtccaagatcagccagagcaccgccagcatcaacgagaacgtgaacgagaagtgcaagttcaccctgccccccctgaagatccacgagtgcaacatcagctgccccaaccccctgcccttccgggagtaccggccccagaccgagggcgtgagcaacctggtcggcctgcccaacaacatctgcctgcagaaaaccagcaaccagatcctgaagcccaagctcatttcctacaccctgcccgtggtgggccagagcggcacctgcatcaccgaccccctgctggccatggacgagggctacttcgcctacagccacctggaacggatcggcagctgcagcaggggcgtgtccaagcagcggatcatcggcgtgggcgaggtgctggaccggggcgacgaggtgcccagcctgttcatgaccaacgtgtggaccccccccaaccccaacaccgtgtaccactgcagcgccgtgtacaacaacgagttctactacgtgctgtgcgccgtgagcaccgtgggcgaccccatcctgaacagcacctactggtccggcagcctgatgatgacccggctggccgtgaagcctaagagcaatggcggcggatacaaccagcaccagctggccctgcggagcatcgagaagggcagatacgacaaagtgatgccctacggccccagcggcatcaagcagggcgacacactgtacttccccgccgtgggcttcctggtccggaccgagttcaagtacaacgacagcaactgccccatcaccaagtgccagtacagcaagcccgagaactgcagactgagcatgggcatccggcccaacagccactacatcctgcggagcggcctgctgaagtacaacctgagcgacggcgagaaccccaaagtcgtctttattgagatcagcgaccagcggctgtccatcggcagccccagcaagatctacgacagcctgggccagcccgtgttctaccaggccagcttcagctgggacaccatgatcaagttcggcgacgtgctgaccgtgaaccccctggtggtgaactggcggaacaataccgtgatcagcagacccggccagagccagtgcccccggttcaacacctgccccgcgatctgcgcggagggcgtgtacaacgacgccttcctgatcgaccggatcaactggatctctgccggcgtgttcctggactccaacgcgaccgccgcgaatcccgtgttcaccgtgtttaaggacaacgagatcctgtaccgggcccagctggccagcgaggacaccaacgcccagaaaaccatcaccaactgctttctgctgaagaacaagatctggtgcatcagcctggtggagatctacgataccggcgacaacgtgatcaggcccaagctgttcgccgtgaagatccccgagcagtgcaccggtggaggtggctctggtggaggaggctctggaggtggtggatcagcggcccagccggcccaggtgcagctggtgcagagcggagccgaggataagaaacctggcgctagcgtgaaggtgtcctgcaaggccagcggcttcaacatcaaggacacctacatccactgggtgcgccaggctccaggacagggcctggaatggatgggccggatcgaccccgccaacgacaacaccctgtacgccagcaagttccagggcagagtgaccatcaccgccgacaccagcagcaacaccgcctacatggaactgagcagcctgagaagcgaggacaccgccgtgtactactgtggcagaggctacggctactacgtgttcgaccactggggccagggcaccaccgtgacagtgtctagcggcggaggcggaagtggaggcggaggaagcggaggcggcggatccgacatcgtgatgacccagagccctagcagcctgtctgccagcgtgggcgaccgcgtgaccattacctgccggaccagccggtccatcagccagtacctggcctggtatcaggaaaagcccggcaaggcccccaagctgctgatctacagcggcagcaccctgcagagcggcgtgccaagcagattcagcggcagcggctccggcaccgacttcaccctgaccatcagcagcctgcagcccgaggacttcgccacctactactgccagcagcacaacgagaaccccctgaccttcgggcagggaacaaaggtggagatcaagagagcggccgcaagaggttctcatcaccatcaccatcactaa

SEQ ID NO: 4 - protein, 842 aa, synthetic construct
  REGION 1..842: note = Synthetic Construct
MKKINEGLLDSKILSAFNTVIALLGSIVIIVMNIMIIQNYTRSTDNQAVIKDALQGIQQQIKGLADKIGTEIGPKVSLIDTSSTITIPANIGLLGSKISQSTASINENVNEKCKFTLPPLKIHECNISCPNPLPFREYRPQTEGVSNLVGLPNNICLQKTSNQILKPKLISYTLPVVGQSGTCITDPLLAMDEGYFAYSHLERIGSCSRGVSKQRIIGVGEVLDRGDEVPSLFMTNVWTPPNPNTVYHCSAVYNNEFYYVLCAVSTVGDPILNSTYWSGSLMMTRLAVKPKSNGGGYNQHQLALRSIEKGRYDKVMPYGPSGIKQGDTLYFPAVGFLVRTEFKYNDSNCPITKCQYSKPENCRLSMGIRPNSHYILRSGLLKYNLSDGENPKVVFIEISDQRLSIGSPSKIYDSLGQPVFYQASFSWDTMIKFGDVLTVNPLVVNWRNNTVISRPGQSQCPRFNTCPAICAEGVYNDAFLIDRINWISAGVFLDSNATAANPVFTVFKDNEILYRAQLASEDTNAQKTITNCFLLKNKIWCISLVEIYDTGDNVIRPKLFAVKIPEQCTGGGGSGGGGSGGGGSAAQPAQVQLVQSGAEDKKPGASVKVSCKASGFNIKDTYIHWVRQAPGQGLEWMGRIDPANDNTLYASKFQGRVTITADTSSNTAYMELSSLRSEDTAVYYCGRGYGYYVFDHWGQGTTVTVSSGGGGSGGGGSGGGGSDIVMTQSPSSLSASVGDRVTITCRTSRSISQYLAWYQEKPGKAPKLLIYSGSTLQSGVPSRFSGSGSGTDFTLTISSLQPEDFATYYCQQHNENPLTFGQGTKVEIKRAAARGSHHHHHH

SEQ ID NO: 5 - DNA, 2211 bp, synthetic construct
  misc_feature 1..2211: note = Truncated and mutated (E501A, W504A, Q530A, E533A) NiV G protein(GcDelta34) fused to IL-7
  source 1..2211: mol_type = other DNA
  CDS 1..2211
atgaagaagatcaacgagggcctgctggacagcaagatcctgagcgccttcaacaccgtgatcgccctgctgggcagcatcgtgatcattgtgatgaacatcatgatcatccagaactacaccagaagcaccgacaaccaggccgtgatcaaggacgctctccaggggatccagcagcagatcaagggcctggccgacaagatcggcaccgagatcggccccaaggtgtccctgatcgacaccagcagcaccatcaccatccccgccaacatcggcctgctggggtccaagatcagccagagcaccgccagcatcaacgagaacgtgaacgagaagtgcaagttcaccctgccccccctgaagatccacgagtgcaacatcagctgccccaaccccctgcccttccgggagtaccggccccagaccgagggcgtgagcaacctggtcggcctgcccaacaacatctgcctgcagaaaaccagcaaccagatcctgaagcccaagctcatttcctacaccctgcccgtggtgggccagagcggcacctgcatcaccgaccccctgctggccatggacgagggctacttcgcctacagccacctggaacggatcggcagctgcagcaggggcgtgtccaagcagcggatcatcggcgtgggcgaggtgctggaccggggcgacgaggtgcccagcctgttcatgaccaacgtgtggaccccccccaaccccaacaccgtgtaccactgcagcgccgtgtacaacaacgagttctactacgtgctgtgcgccgtgagcaccgtgggcgaccccatcctgaacagcacctactggtccggcagcctgatgatgacccggctggccgtgaagcctaagagcaatggcggcggatacaaccagcaccagctggccctgcggagcatcgagaagggcagatacgacaaagtgatgccctacggccccagcggcatcaagcagggcgacacactgtacttccccgccgtgggcttcctggtccggaccgagttcaagtacaacgacagcaactgccccatcaccaagtgccagtacagcaagcccgagaactgcagactgagcatgggcatccggcccaacagccactacatcctgcggagcggcctgctgaagtacaacctgagcgacggcgagaaccccaaagtcgtctttattgagatcagcgaccagcggctgtccatcggcagccccagcaagatctacgacagcctgggccagcccgtgttctaccaggccagcttcagctgggacaccatgatcaagttcggcgacgtgctgaccgtgaaccccctggtggtgaactggcggaacaataccgtgatcagcagacccggccagagccagtgcccccggttcaacacctgccccgcgatctgcgcggagggcgtgtacaacgacgccttcctgatcgaccggatcaactggatctctgccggcgtgttcctggactccaacgcgaccgccgcgaatcccgtgttcaccgtgtttaaggacaacgagatcctgtaccgggcccagctggccagcgaggacaccaacgcccagaaaaccatcaccaactgctttctgctgaagaacaagatctggtgcatcagcctggtggagatctacgataccggcgacaacgtgatcaggcccaagctgttcgccgtgaagatccccgagcagtgcaccggtatggccgattgtgatattgaaggtaaagatggcaaacaatatgagagtgttctaatggtcagcatcgatcaattattggacagcatgaaagaaattggtagcaattgcctgaataatgaatttaacttttttaaaagacatatctgtgatgctaataaggaaggtatgtttttattccgtgctgctcgcaagttgaggcaatttcttaaaatgaatagcactggtgattttgatctccacttattaaaagtttcagaaggcacaacaatactgttgaactgcactggccaggttaaaggaagaaaaccagctgccctgggtgaagcccaaccaacaaagagtttggaagaaaataaatctttaaaggaacagaaaaaactgaatgacttgtgtttcctaaagagactattacaagagataaaaacttgttggaataaaattttgatgggcactaaagaacacgcggccgcaagaggttctcatcaccatcaccatcactaa

SEQ ID NO: 6 - protein, 736 aa, synthetic construct
  REGION 1..736: note = Synthetic Construct
MKKINEGLLDSKILSAFNTVIALLGSIVIIVMNIMIIQNYTRSTDNQAVIKDALQGIQQQIKGLADKIGTEIGPKVSLIDTSSTITIPANIGLLGSKISQSTASINENVNEKCKFTLPPLKIHECNISCPNPLPFREYRPQTEGVSNLVGLPNNICLQKTSNQILKPKLISYTLPVVGQSGTCITDPLLAMDEGYFAYSHLERIGSCSRGVSKQRIIGVGEVLDRGDEVPSLFMTNVWTPPNPNTVYHCSAVYNNEFYYVLCAVSTVGDPILNSTYWSGSLMMTRLAVKPKSNGGGYNQHQLALRSIEKGRYDKVMPYGPSGIKQGDTLYFPAVGFLVRTEFKYNDSNCPITKCQYSKPENCRLSMGIRPNSHYILRSGLLKYNLSDGENPKVVFIEISDQRLSIGSPSKIYDSLGQPVFYQASFSWDTMIKFGDVLTVNPLVVNWRNNTVISRPGQSQCPRFNTCPAICAEGVYNDAFLIDRINWISAGVFLDSNATAANPVFTVFKDNEILYRAQLASEDTNAQKTITNCFLLKNKIWCISLVEIYDTGDNVIRPKLFAVKIPEQCTGMADCDIEGKDGKQYESVLMVSIDQLLDSMKEIGSNCLNNEFNFFKRHICDANKEGMFLFRAARKLRQFLKMNSTGDFDLHLLKVSEGTTILLNCTGQVKGRKPAALGEAQPTKSLEENKSLKEQKKLNDLCFLKRLLQEIKTCWNKILMGTKEHAAARGSHHHHHH

SEQ ID NO: 7 - DNA, 2229 bp, synthetic construct
  misc_feature 1..2229: note = Truncated and mutated (E501A, W504A, Q530A, E533A) NiV G protein(GcDelta34) fused to a designed ankaryin repeat protein (DARPin)directed against human EpCAM
  source 1..2229: mol_type = other DNA
  CDS 1..2229
atgaagaagatcaacgagggcctgctggacagcaagatcctgagcgccttcaacaccgtgatcgccctgctgggcagcatcgtgatcattgtgatgaacatcatgatcatccagaactacaccagaagcaccgacaaccaggccgtgatcaaggacgctctccaggggatccagcagcagatcaagggcctggccgacaagatcggcaccgagatcggccccaaggtgtccctgatcgacaccagcagcaccatcaccatccccgccaacatcggcctgctggggtccaagatcagccagagcaccgccagcatcaacgagaacgtgaacgagaagtgcaagttcaccctgccccccctgaagatccacgagtgcaacatcagctgccccaaccccctgcccttccgggagtaccggccccagaccgagggcgtgagcaacctggtcggcctgcccaacaacatctgcctgcagaaaaccagcaaccagatcctgaagcccaagctcatttcctacaccctgcccgtggtgggccagagcggcacctgcatcaccgaccccctgctggccatggacgagggctacttcgcctacagccacctggaacggatcggcagctgcagcaggggcgtgtccaagcagcggatcatcggcgtgggcgaggtgctggaccggggcgacgaggtgcccagcctgttcatgaccaacgtgtggaccccccccaaccccaacaccgtgtaccactgcagcgccgtgtacaacaacgagttctactacgtgctgtgcgccgtgagcaccgtgggcgaccccatcctgaacagcacctactggtccggcagcctgatgatgacccggctggccgtgaagcctaagagcaatggcggcggatacaaccagcaccagctggccctgcggagcatcgagaagggcagatacgacaaagtgatgccctacggccccagcggcatcaagcagggcgacacactgtacttccccgccgtgggcttcctggtccggaccgagttcaagtacaacgacagcaactgccccatcaccaagtgccagtacagcaagcccgagaactgcagactgagcatgggcatccggcccaacagccactacatcctgcggagcggcctgctgaagtacaacctgagcgacggcgagaaccccaaagtcgtctttattgagatcagcgaccagcggctgtccatcggcagccccagcaagatctacgacagcctgggccagcccgtgttctaccaggccagcttcagctgggacaccatgatcaagttcggcgacgtgctgaccgtgaaccccctggtggtgaactggcggaacaataccgtgatcagcagacccggccagagccagtgcccccggttcaacacctgccccgcgatctgcgcggagggcgtgtacaacgacgccttcctgatcgaccggatcaactggatctctgccggcgtgttcctggactccaacgcgaccgccgcgaatcccgtgttcaccgtgtttaaggacaacgagatcctgtaccgggcccagctggccagcgaggacaccaacgcccagaaaaccatcaccaactgctttctgctgaagaacaagatctggtgcatcagcctggtggagatctacgataccggcgacaacgtgatcaggcccaagctgttcgccgtgaagatccccgagcagtgcaccggtgacctgggtaagaaactgctggaagctgctcgtgctggtcaggacgacgaagttcgtatcctgatggctaacggtgctgacgttaacgctaaggacgagtatggttctactccgctgcacctagctgctactcttggtcacctggaaatcgttgaagttctgctgaagcacggtgctgacgttaacgctgatgacgctactggtcttactccgctgcacctggctgcttggaatggtcacctggagatcgttgaagttctgctgaagtacggtgctgacgttaacgctatggactttgagggttggactccgctgcacctggctgctcattttggtcacctggaaatcgttgaagttctgctgaagtacggtgctgacgttaacgctcaggacaaattcggtaagaccccgttcgacctagcgatcgacaacggtaacgaggacattgctgaagtgctgcaaaaagcggcgaagcttaatgcggccgcaagaggttctcatcaccatcaccatcactaa

SEQ ID NO: 8 - protein, 742 aa, synthetic construct
  REGION 1..742: note = Synthetic Construct
MKKINEGLLDSKILSAFNTVIALLGSIVIIVMNIMIIQNYTRSTDNQAVIKDALQGIQQQIKGLADKIGTEIGPKVSLIDTSSTITIPANIGLLGSKISQSTASINENVNEKCKFTLPPLKIHECNISCPNPLPFREYRPQTEGVSNLVGLPNNICLQKTSNQILKPKLISYTLPVVGQSGTCITDPLLAMDEGYFAYSHLERIGSCSRGVSKQRIIGVGEVLDRGDEVPSLFMTNVWTPPNPNTVYHCSAVYNNEFYYVLCAVSTVGDPILNSTYWSGSLMMTRLAVKPKSNGGGYNQHQLALRSIEKGRYDKVMPYGPSGIKQGDTLYFPAVGFLVRTEFKYNDSNCPITKCQYSKPENCRLSMGIRPNSHYILRSGLLKYNLSDGENPKVVFIEISDQRLSIGSPSKIYDSLGQPVFYQASFSWDTMIKFGDVLTVNPLVVNWRNNTVISRPGQSQCPRFNTCPAICAEGVYNDAFLIDRINWISAGVFLDSNATAANPVFTVFKDNEILYRAQLASEDTNAQKTITNCFLLKNKIWCISLVEIYDTGDNVIRPKLFAVKIPEQCTGDLGKKLLEAARAGQDDEVRILMANGADVNAKDEYGSTPLHLAATLGHLEIVEVLLKHGADVNADDATGLTPLHLAAWNGHLEIVEVLLKYGADVNAMDFEGWTPLHLAAHFGHLEIVEVLLKYGADVNAQDKFGKTPFDLAIDNGNEDIAEVLQKAAKLNAAARGSHHHHHH

SEQ ID NO: 9 - protein, 602 aa, Nipah virus
MPAENKKVRFENTTSDKGKIPSKVIKSYYGTMDIKKINEGLLDSKILSAFNTVIALLGSIVIIVMNIMIIQNYTRSTDNQAVIKDALQGIQQQIKGLADKIGTEIGPKVSLIDTSSTITIPANIGLLGSKISQSTASINENVNEKCKFTLPPLKIHECNISCPNPLPFREYRPQTEGVSNLVGLPNNICLQKTSNQILKPKLISYTLPVVGQSGTCITDPLLAMDEGYFAYSHLERIGSCSRGVSKQRIIGVGEVLDRGDEVPSLFMTNVWTPPNPNTVYHCSAVYNNEFYYVLCAVSTVGDPILNSTYWSGSLMMTRLAVKPKSNGGGYNQHQLALRSIEKGRYDKVMPYGPSGIKQGDTLYFPAVGFLVRTEFKYNDSNCPITKCQYSKPENCRLSMGIRPNSHYILRSGLLKYNLSDGENPKVVFIEISDQRLSIGSPSKIYDSLGQPVFYQASFSWDTMIKFGDVLTVNPLVVNWRNNTVISRPGQSQCPRFNTCPEICWEGVYNDAFLIDRINWISAGVFLDSNQTAENPVFTVFKDNEILYRAQLASEDTNAQKTITNCFLLKNKIWCISLVEIYDTGDNVIRPKLFAVKIPEQCT

SEQ ID NO: 10 - protein, 617 aa, Measles virus
MSPQRDRINAFYKDNPHPKGSRIVINREHLMIDRPYVLLAVLFVMFLSLIGLLAIAGIRLHRAAIYTAEIHKSLSTNLDVTNSIEHQVKDVLTPLFKIIGDEVGLRTPQRFTDLVKFISDKIKFLNPDREYDFRDLTWCINPPERIKLDYDQYCADVAAEELMNALVNSTLLETRTTNQFLAVSKGNCSGPTTIRGQFSNMSLSLLDLYLGRGYNVSSIVTMTSQGMYGGTYLVEKPNLSSKRSELSQLSMYRVFEVGVIRNPGLGAPVFHMTNYLEQPVSNDLSNCMVALGELKLAALCHGEDSITIPYQGSGKGVSFQLVKLGVWKSPTDMQSWVPLSTDDPVIDRLYLSSHRGVIADNQAKWAVPTTRTDDKLRMETCFQQACKGKIQALCENPEWAPLKDNRIPSYGVLSVDLSLTVELKIKIASGFGPLITHGSGMDLYKSNHNNVYWLTIPPMKNLALGVINTLEWIPRFKVSPYLFTVPIKEAGGDCHAPTYLPAEVDGDVKLSSNLVILPGQDLQYVLATYDTSRVEHAVVYYVYSPSRSFSYFYPFRLPIKGVPIELQVECFTWDQKLWCRHFCVLADSESGGHITHSGMVGMGVSCTVTREDGTNRR

SEQ ID NO: 11 - protein, 546 aa, Nipah virus
MVVILDKRCYCNLLILILMISECSVGILHYEKLSKIGLVKGVTRKYKIKSNPLTKDIVIKMIPNVSNMSQCTGSVMENYKTRLNGILTPIKGALEIYKNNTHDLVGDVRLAGVIMAGVAIGIATAAQITAGVALYEAMKNADNINKLKSSIESTNEAVVKLQETAEKTVYVLTALQDYINTNLVPTIDKISCKQTELSLDLALSKYLSDLLFVFGPNLQDPVSNSMTIQAISQAFGGNYETLLRTLGYATEDFDDLLESDSITGQIIYVDLSSYYIIVRVYFPILTEIQQAYIQELLPVSFNNDNSEWISIVPNFILVRNTLISNIEIGFCLITKRSVICNQDYATPMTNNMRECLTGSTEKCPRELVVSSHVPRFALSNGVLFANCISVTCQCQTTGRAISQSGEQTLLMIDNTTCPTAVLGNVIISLGKYLGSVNYNSEGIAIGPPVFTDKVDISSQISSMNQSLQQSKDYIKEAQRLLDTVNPSLISMLSMIILYVLSIASLCIGLITFISFIIVEKKRNTYSRLEDRRVRPTSSGDLYYIGT

SEQ ID NO: 12 - protein, 553 aa, Measles virus
MSIMGLKVNVSAIFMAVLLTLQTPTGQIHWGNLSKIGVVGIGSASYKVMTRSSHQSLVIKLMPNITLLNNCTRVEIAEYRRLLRTVLEPIRDALNAMTQNIRPVQSVASSRRHKRFAGVVLAGAALGVATAAQITAGIALHQSMLNSQAIDNLRASLETTNQAIEAIRQAGQEMILAVQGVQDYINNELIPSMNQLSCDLIGQKLGLKLLRYYTEILSLFGPSLRDPISAEISIQALSYALGGDINKVLEKLGYSGGDLLGILESRGIKARITHVDTESYFIVLSIAYPTLSEIKGVIVHRLEGVSYNIGSQEWYTTVPKYVATQGYLISNFDESSCTFMPEGTVCSQNALYPMSPLLQECLRGSTKSCARTLVSGSFGNRFILSQGNLIANCASILCKCYTTGTIINQDPDKILTYIAADHCPVVEVNGVTIQVGSRRYPDAVYLHRIDLGPPISLERLDVGTNLGNAIAKLEDAKELLESSDQILRSMKGLSSTSIVYILIAVCLGGLIGIPALICCCRGRCNKKGEQVGMSRPGLKPDLTGTSKSYVRSL

SEQ ID NO: 13 - DNA, 2328 bp, synthetic construct
  misc_feature 1..2328: note = Truncated and mutated (Y481A, R533A, S548L, F549S) MeV H protein(Hcdelta15) fused to IL-17
  source 1..2328: mol_type = other DNA
  CDS 1..2328
atgcatcccaagggaagtaggatagtcattaacagagaacatcttatgattgatagaccttatgttttgctggctgttctgtttgtcatgtttctgagcttgatcgggttgctagccattgcaggcattagacttcatcgggcagccatctacaccgcagagatccataaaagcctcagcaccaatctagatgtaactaactcaatcgagcatcaggtcaaggacgtgctgacaccactcttcaaaatcatcggtgatgaagtgggcctgaggacacctcagagattcactgacctagtgaaattcatctctgacaagattaaattccttaatccggatagggagtacgacttcagagatctcacttggtgtatcaacccgccagagagaatcaaattggattatgatcaatactgtgcagatgtggctgctgaagagctcatgaatgcattggtgaactcaactctactggagaccagaacaaccaatcagttcctagctgtctcaaagggaaactgctcagggcccactacaatcagaggtcaattctcaaacatgtcgctgtccctgttagacttgtatttaggtcgaggttacaatgtgtcatctatagtcactatgacatcccagggaatgtatgggggaacttacctagtggaaaagcctaatctgagcagcaaaaggtcagagttgtcacaactgagcatgtaccgagtgtttgaagtaggtgttatcagaaatccgggtttgggggctccggtgttccatatgacaaactatcttgagcaaccagtcagtaatgatctcagcaactgtatggtggctttgggggagctcaaactcgcagccctttgtcacggggaagattctatcacaattccctatcagggatcagggaaaggtgtcagcttccagctcgtcaagctaggtgtctggaaatccccaaccgacatgcaatcctgggtccccttatcaacggatgatccagtgatagacaggctttacctctcatctcacagaggtgttatcgctgacaatcaagcaaaatgggctgtcccgacaacacgaacagatgacaagttgcgaatggagacatgcttccaacaggcgtgtaagggtaaaatccaagcactctgcgagaatcccgagtgggcaccattgaaggataacaggattccttcatacggggtcttgtctgttgatctgagtctgacagttgagcttaaaatcaaaattgcttcgggattcgggccattgatcacacacggttcagggatggacctatacaaatccaaccacaacaatgtgtattggctgactatcccgccaatgaagaacctagccttaggtgtaatcaacacattggagtggataccgagattcaaggttagtcccgcgctcttcaatgtcccaattaaggaagcaggcgaagactgccatgccccaacatacctacctgcggaggtggatggtgatgtcaaactcagttccaatctggtgattctacctggtcaagatctccaatatgttttggcaacctacgatacttccgcggttgaacatgctgtggtttattacgtttacagcccaagccgctcattttcttacttttatccttttaggttgcctataaagggggtccccatcgaattacaagtggaatgcttcacatgggaccaaaaactctggtgccgtcacttctgtgtgcttgcggactcagaatctggtggacatatcactcactctgggatggagggcatgggagtcagctgcacagtcacccgggaagatggaaccaatatcgagggaagggcggcccagccggccatggccgattgtgatattgaaggtaaagatggcaaacaatatgagagtgttctaatggtcagcatcgatcaattattggacagcatgaaagaaattggtagcaattgcctgaataatgaatttaacttttttaaaagacatatctgtgatgctaataaggaaggtatgtttttattccgtgctgctcgcaagttgaggcaatttcttaaaatgaatagcactggtgattttgatctccacttattaaaagtttcagaaggcacaacaatactgttgaactgcactggccaggttaaaggaagaaaaccagctgccctgggtgaagcccaaccaacaaagagtttggaagaaaataaatctttaaaggaacagaaaaaactgaatgacttgtgtttcctaaagagactattacaagagataaaaacttgttggaataaaattttgatgggcactaaagaacacgcggccgcaagaggatcgcatcaccatcaccatcactga

SEQ ID NO: 14 - protein, 775 aa, synthetic construct
  REGION 1..775: note = Synthetic Construct
MHPKGSRIVINREHLMIDRPYVLLAVLFVMFLSLIGLLAIAGIRLHRAAIYTAEIHKSLSTNLDVTNSIEHQVKDVLTPLFKIIGDEVGLRTPQRFTDLVKFISDKIKFLNPDREYDFRDLTWCINPPERIKLDYDQYCADVAAEELMNALVNSTLLETRTTNQFLAVSKGNCSGPTTIRGQFSNMSLSLLDLYLGRGYNVSSIVTMTSQGMYGGTYLVEKPNLSSKRSELSQLSMYRVFEVGVIRNPGLGAPVFHMTNYLEQPVSNDLSNCMVALGELKLAALCHGEDSITIPYQGSGKGVSFQLVKLGVWKSPTDMQSWVPLSTDDPVIDRLYLSSHRGVIADNQAKWAVPTTRTDDKLRMETCFQQACKGKIQALCENPEWAPLKDNRIPSYGVLSVDLSLTVELKIKIASGFGPLITHGSGMDLYKSNHNNVYWLTIPPMKNLALGVINTLEWIPRFKVSPALFNVPIKEAGEDCHAPTYLPAEVDGDVKLSSNLVILPGQDLQYVLATYDTSAVEHAVVYYVYSPSRSFSYFYPFRLPIKGVPIELQVECFTWDQKLWCRHFCVLADSESGGHITHSGMEGMGVSCTVTREDGTNIEGRAAQPAMADCDIEGKDGKQYESVLMVSIDQLLDSMKEIGSNCLNNEFNFFKRHICDANKEGMFLFRAARKLRQFLKMNSTGDFDLHLLKVSEGTTILLNCTGQVKGRKPAALGEAQPTKSLEENKSLKEQKKLNDLCFLKRLLQEIKTCWNKILMGTKEHAAARGSHHHHHH

SEQ ID NO: 15 - protein, 523 aa, synthetic construct
  REGION 1..523: note = Truncated MeV fusion glycoprotein (FcDelta30)
MSIMGLKVNVSAIFMAVLLTLQTPTGQIHWGNLSKIGVVGIGSASYKVMTRSSHQSLVIKLMPNITLLNNCTRVEIAEYRRLLRTVLEPIRDALNAMTQNIRPVQSVASSRRHKRFAGVVLAGAALGVATAAQITAGIALHQSMLNSQAIDNLRASLETTNQAIEAIRQAGQEMILAVQGVQDYINNELIPSMNQLSCDLIGQKLGLKLLRYYTEILSLFGPSLRDPISAEISIQALSYALGGDINKVLEKLGYSGGDLLGILESRGIKARITHVDTESYFIVLSIAYPTLSEIKGVIVHRLEGVSYNIGSQEWYTTVPKYVATQGYLISNFDESSCTFMPEGTVCSQNALYPMSPLLQECLRGSTKSCARTLVSGSFGNRFILSQGNLIANCASILCKCYTTGTIINQDPDKILTYIAADHCPVVEVNGVTIQVGSRRYPDAVYLHRIDLGPPISLERLDVGTNLGNAIAKLEDAKELLESSDQILRSMKGLSSTSIVYILIAVCLGGLIGIPALICCCRGR

SEQ ID NO: 16 - protein, 524 aa, synthetic construct
  REGION 1..524: note = Truncated NiV fusion glycoprotein (FcDelta22)
MVVILDKRCYCNLLILILMISECSVGILHYEKLSKIGLVKGVTRKYKIKSNPLTKDIVIKMIPNVSNMSQCTGSVMENYKTRLNGILTPIKGALEIYKNNTHDLVGDVRLAGVIMAGVAIGIATAAQITAGVALYEAMKNADNINKLKSSIESTNEAVVKLQETAEKTVYVLTALQDYINTNLVPTIDKISCKQTELSLDLALSKYLSDLLFVFGPNLQDPVSNSMTIQAISQAFGGNYETLLRTLGYATEDFDDLLESDSITGQIIYVDLSSYYIIVRVYFPILTEIQQAYIQELLPVSFNNDNSEWISIVPNFILVRNTLISNIEIGFCLITKRSVICNQDYATPMTNNMRECLTGSTEKCPRELVVSSHVPRFALSNGVLFANCISVTCQCQTTGRAISQSGEQTLLMIDNTTCPTAVLGNVIISLGKYLGSVNYNSEGIAIGPPVFTDKVDISSQISSMNQSLQQSKDYIKEAQRLLDTVNPSLISMLSMIILYVLSIASLCIGLITFISFIIVEKKRNT